European Patent Application EP 4 389 890 A1, published June 26, 2024. Title: tRNA, aminoacyl tRNA, reagent for synthesizing polypeptide, method for introducing non-natural amino acid, method for producing polypeptide, method for producing nucleic acid display library, nucleic acid-polypeptide conjugate, and screening method. Applicant: FUJIFILM Corporation. The sequence listing filed with the application follows.

SEQUENCE LISTING (21 sequences)

SEQ ID NO: 1 - RNA, 75 nt, synthetic construct
  misc_feature 1..75: note = tRNA
  misc_feature 33..35: note = anticodon UUA
  source 1..75: mol_type = other RNA
gggagagtagttcaatggtagaacgtcggtctttaaaaccgagcgttgagggttcgattcctttctctcccacca

SEQ ID NO: 2 - RNA, 74 nt, synthetic construct
  misc_feature 1..74: note = tRNA
  misc_feature 33..35: note = anticodon UUA
  source 1..74: mol_type = other RNA
gggggtgtagtttagtggcagaacaacagtctttaaaactgtctgtgtgggttcgattccttccacccccacca

SEQ ID NO: 3 - RNA, 74 nt, synthetic construct
  misc_feature 1..74: note = tRNA
  misc_feature 33..35: note = anticodon UUA
  source 1..74: mol_type = other RNA
gggggcatagttcaacggtagaatagaggtctttaaaacctttggtgtgggttcgattcctactgcccccacca

SEQ ID NO: 4 - RNA, 77 nt, synthetic construct
  misc_feature 1..77: note = tRNA
  misc_feature 35..37: note = anticodon UUA
  source 1..77: mol_type = other RNA
gggggtgtagttccaattggtagaacagcggtctttaaaaccgatggttgcgggttcgagtcctgccacccccacca

SEQ ID NO: 5 - RNA, 74 nt, synthetic construct
  misc_feature 1..74: note = tRNA
  misc_feature 33..35: note = anticodon UUA
  source 1..74: mol_type = other RNA
ggcggtgtagtttagtggcagaacaacagtctttaaaactgtctgtgtgggttcgattccttccaccgccacca

SEQ ID NO: 6 - RNA, 74 nt, synthetic construct
  misc_feature 1..74: note = tRNA
  misc_feature 33..35: note = anticodon UUA
  source 1..74: mol_type = other RNA
ggaggtgtagtttagtggcagaacaacagtctttaaaactgtctgtgtgggttcgattccttccacctccacca

SEQ ID NO: 7 - RNA, 74 nt, synthetic construct
  misc_feature 1..74: note = tRNA
  misc_feature 33..35: note = anticodon UUA
  source 1..74: mol_type = other RNA
ggtggtgtagtttagtggcagaacaacagtctttaaaactgtctgtgtgggttcgattccttccaccaccacca

SEQ ID NO: 8 - RNA, 74 nt, synthetic construct
  misc_feature 1..74: note = tRNA
  misc_feature 33..35: note = anticodon UUA
  source 1..74: mol_type = other RNA
gggggtgtagtttagtggcagaacaacagtctttaaaactgtctgtgtgggttcgattccttccacctccacca

SEQ ID NO: 9 - RNA, 74 nt, synthetic construct
  misc_feature 1..74: note = tRNA
  misc_feature 33..35: note = anticodon UUA
  source 1..74: mol_type = other RNA
ggtggtgtagtttagtggcagaacaacagtctttaaaactgtctgtgtgggttcgattccttccaccgccacca

SEQ ID NO: 10 - RNA, 74 nt, synthetic construct
  misc_feature 1..74: note = tRNA
  misc_feature 33..35: note = anticodon UUA
  source 1..74: mol_type = other RNA
gggcgtgtagtttagtggcagaacaacagtctttaaaactgtctgtgtgggttcgattccttccacgcccacca

SEQ ID NO: 11 - RNA, 74 nt, synthetic construct
  misc_feature 1..74: note = tRNA
  misc_feature 33..35: note = anticodon UUA
  source 1..74: mol_type = other RNA
gggagtgtagtttagtggcagaacaacagtctttaaaactgtctgtgtgggttcgattccttccactcccacca

SEQ ID NO: 12 - RNA, 74 nt, synthetic construct
  misc_feature 1..74: note = tRNA
  misc_feature 33..35: note = anticodon UUA
  source 1..74: mol_type = other RNA
gggtgtgtagtttagtggcagaacaacagtctttaaaactgtctgtgtgggttcgattccttccacacccacca

SEQ ID NO: 13 - RNA, 74 nt, synthetic construct
  misc_feature 1..74: note = tRNA
  misc_feature 33..35: note = anticodon UUA
  source 1..74: mol_type = other RNA
gggggtgtagtttagtggcagaacaacagtctttaaaactgtctgtgtgggttcgattccttccactcccacca

SEQ ID NO: 14 - RNA, 74 nt, synthetic construct
  misc_feature 1..74: note = tRNA
  misc_feature 33..35: note = anticodon UUA
  source 1..74: mol_type = other RNA
gggtgtgtagtttagtggcagaacaacagtctttaaaactgtctgtgtgggttcgattccttccacgcccacca

SEQ ID NO: 15 - RNA, 74 nt, synthetic construct
  misc_feature 1..74: note = tRNA
  misc_feature 33..35: note = anticodon UUA
  source 1..74: mol_type = other RNA
gggggtgtagtttagtggcagaacaacagtctttaaaactgtctgtgtgggttcgattccttccacccccgcca

SEQ ID NO: 16 - RNA, 74 nt, synthetic construct
  misc_feature 1..74: note = tRNA
  misc_feature 33..35: note = anticodon UUA
  source 1..74: mol_type = other RNA
ggtggtgtagtttagtggcagaacaacagtctttaaaactgtctgtgtgggttcgattccttccaccgccgcca

SEQ ID NO: 17 - RNA, 74 nt, synthetic construct
  misc_feature 1..74: note = tRNA
  misc_feature 33..35: note = anticodon UUA
  source 1..74: mol_type = other RNA
gggggtgtagtttagtggcagaacaacagtctttaaaactgtctgtgtgggttcgattccttccactcccgcca

SEQ ID NO: 18 - RNA, 74 nt, Mycoplasma pneumoniae
  misc_feature 1..74: note = tRNA
  misc_feature 33..35: note = anticodon CCA
  source 1..74: mol_type = tRNA
gggggtgtagtttagtggcagaacaacagtctccaaaactgtctgtgtgggttcgattccttccacccccgcca

SEQ ID NO: 19 - RNA, 75 nt, synthetic construct
  misc_feature 1..75: note = tRNA
  misc_feature 33..35: note = anticodon CUA
  source 1..75: mol_type = other RNA
gggagagtagttcaatggtagaacgtcggtctctaaaaccgagcgttgagggttcgattcctttctctcccacca

SEQ ID NO: 20 - protein, 20 aa, synthetic construct
  REGION 1..20: note = Translation product
  SITE 4: note = nonnatural amino acid
MCKXKPRSKNMSDYKDDDDK

SEQ ID NO: 21 - DNA, 60 bp, synthetic construct
  misc_feature 1..60: note = Synthetic oligonucleotide
  misc_feature 10..12: note = taa is a triplet to be translated
  source 1..60: mol_type = other DNA
atgtgcaaataaaaaccgcggagcaaaaacatgagcgattataaagatgatgatgataag